European Patent Application EP 4 400 110 A1, published July 17, 2024. Title: AGENT AND KIT FOR INHIBITING PROGRESSION OF OSTEOARTHRITIS. Applicant: KYUSHU UNIVERSITY, NATIONAL UNIVERSITY CORPORATION. Application JP. The sequence listing filed with the application follows.

SEQUENCE LISTING (8 sequences)

SEQ ID NO: 1 - DNA, 21 bp, synthetic construct
  misc_feature 1..21: note = synthetic nucleotide used for qPCR as primer
  source 1..21: mol_type = other DNA
ggtacatcctcgacggcatct

SEQ ID NO: 2 - DNA, 21 bp, synthetic construct
  misc_feature 1..21: note = synthetic nucleotide used for qPCR as primer
  source 1..21: mol_type = other DNA
gtgcctctttgctgctttcac

SEQ ID NO: 3 - DNA, 25 bp, synthetic construct
  misc_feature 1..25: note = synthetic nucleotide used for qPCR as primer
  source 1..25: mol_type = other DNA
gtctctctatggtccaggagatgaa

SEQ ID NO: 4 - DNA, 19 bp, synthetic construct
  misc_feature 1..19: note = synthetic nucleotide used for qPCR as primer
  source 1..19: mol_type = other DNA
aggcgccagaagaatctgt

SEQ ID NO: 5 - DNA, 20 bp, synthetic construct
  misc_feature 1..20: note = synthetic nucleotide used for qPCR as primer
  source 1..20: mol_type = other DNA
aggcactgggctactactat

SEQ ID NO: 6 - DNA, 20 bp, synthetic construct
  misc_feature 1..20: note = synthetic nucleotide used for qPCR as primer
  source 1..20: mol_type = other DNA
gggatagtgaccacattgtt

SEQ ID NO: 7 - DNA, 22 bp, synthetic construct
  misc_feature 1..22: note = synthetic nucleotide used for qPCR as primer
  source 1..22: mol_type = other DNA
ggtgaaggtcggagtcaacgga

SEQ ID NO: 8 - DNA, 22 bp, synthetic construct
  misc_feature 1..22: note = synthetic nucleotide used for qPCR as primer
  source 1..22: mol_type = other DNA
gagggatctcgctcctggaaga